European Patent Specification EP 3 171 886 B1, published June 17, 2026. Title: ANG-(1-7) DERVIATIVE OLIGOPEPTIDES AND METHODS FOR USING AND PRODUCING THE SAME. Applicant: Arizona Board of Regents for the University of Arizona Hay, Meredith Konhilas, John Polt, Robin L. The sequence listing filed with the application follows.

SEQUENCE LISTING (13 sequences)

SEQ ID NO: 1 - protein, 8 aa, Artificial Sequence
  Artificial Construct
  MISC_FEATURE (1)..(1): aspartic acid, glutamic acid, alanine or a derivative thereof.
  MISC_FEATURE (2)..(2): arginine, histidine, lysine, or a derivative thereof
  MISC_FEATURE (3)..(3): valine, alanine, isoleucine, leucine, or a derivative thereof.
  MISC_FEATURE (4)..(4): tyrosine, phenylalanine, tryptophan, or a derivative thereof.
  MISC_FEATURE (5)..(5): isoleucine, valine, alanine, leucine, or a derivative thereof.
  MISC_FEATURE (6)..(6): histidine, arginine, lysine, or a derivative thereof.
  MISC_FEATURE (7)..(7): proline, glycine, serine, or a derivative thereof.
  MISC_FEATURE (8)..(8): can be absent or is serine, threonine, hydroxyproline, or a derivative thereof
XXXXXXXX

SEQ ID NO: 2 - protein, 7 aa, Homo sapiens
DRVYIHP

SEQ ID NO: 3 - protein, 7 aa, Artificial Sequence
  Artificial Construct
  MISC_FEATURE (1)..(7): D-amino acids in C to N direction
DRVYIHP

SEQ ID NO: 4 - protein, 7 aa, Artificial Sequence
  Artificial Construct
  MISC_FEATURE (1)..(7): L-amino acids in C to N direction
DRVYIHP

SEQ ID NO: 5 - protein, 7 aa, Artificial Sequence
  Artificial Construct
  MISC_FEATURE (1)..(7): D-amino acids from N to C direction
DRVYIHP

SEQ ID NO: 6 - protein, 7 aa, Artificial Sequence
  Artificial Construct
  MISC_FEATURE (7)..(7): -OH of carboxylic acid terminal group is replaced with -NH2 group.
DRVYIHP

SEQ ID NO: 7 - protein, 8 aa, Artificial Sequence
  Artificial Construct
  MISC_FEATURE (8)..(8): -OH of the carboxylic acid terminal is replaced with -NH2
DRVYIHPS

SEQ ID NO: 8 - protein, 8 aa, Artificial Sequence
  Artificial Construct
  MISC_FEATURE (8)..(8): Glucosylated and -OH of the carboxylic acid terminal end is replaced with -NH2.
DRVYIHPS

SEQ ID NO: 9 - protein, 8 aa, Artificial Sequence
  Artificial Construct
  MISC_FEATURE (8)..(8): Lactosylated and -OH of the carboxylic acid terminal group is replaced with -NH2.
DRVYIHPS

SEQ ID NO: 10 - protein, 7 aa, Artificial Sequence
  Artificial Construct
  MISC_FEATURE (7)..(7): Glucosylated and -OH of the terminal carboxylic acid end is replaced with -NH2.
DRVYIHS

SEQ ID NO: 11 - protein, 8 aa, Artificial Sequence
  Artificial Construct
  MISC_FEATURE (2)..(3): Any amino acid residue
  MISC_FEATURE (6)..(6): Any amino acid residue
  MISC_FEATURE (8)..(8): May optionally be glucosylated or lactosylated and -OH of the terminal carboxylic acid end is replaced with -NH2
AXXYIXPS

SEQ ID NO: 12 - protein, 8 aa, Artificial Sequence
  Artificial Construct
  MISC_FEATURE (3)..(3): Any amino acid residue
  MISC_FEATURE (5)..(5): Any amino acid residue
  MISC_FEATURE (8)..(8): May optionally be glucosylated or lactosylated and -OH of the terminal carboxylic acid end is replaced with -NH2
DRXYXHPS

SEQ ID NO: 13 - protein, 8 aa, Artificial Sequence
  Artificial Construct
  MISC_FEATURE (3)..(5): Any amino acid residue
  MISC_FEATURE (8)..(8): May optionally be glucosylated or lactosylated and -OH of the terminal carboxylic acid end is replaced with -NH2
DRXXXHPS